European Patent Application EP 4 123 023 A1, published January 25, 2023. Title: A Hetero Nucleic Acid Comprising A Morpholino Nucleic Acid. Applicant: National University Corporation Tokyo Medical and Dental University. The sequence listing filed with the application follows.

SEQUENCE LISTING (19 sequences)

SEQ ID NO: 1 - DNA, 25 bp, Artificial
  synthetic
  misc_feature (1)..(25): Morpholino nucleic acid
ggccaaacctcggcttacctgaaat

SEQ ID NO: 2 - RNA, 25 nt, Artificial
  synthetic
  misc_feature (1)..(3), (23)..(25): 2'-O-Me RNA
auuucagguaagccgagguuuggcc

SEQ ID NO: 3 - DNA, 21 bp, Artificial
  primer
atccagcagtcagaaagcaaa

SEQ ID NO: 4 - DNA, 21 bp, Artificial
  primer
cagccatccatttctgtaagg

SEQ ID NO: 5 - DNA, 2534 bp, Mus musculus
  SR-B1 mRNA
ggaatcccgcgccgaactcgggggcgggctgcccgggccatggcgcataaagcctctggccacctgcagggctactgctgctccggccaccgccaggcacacaccttgctgctgagggagtctcggcttctgtcatctctgtggcctccgtcacctctgtctccgtctccttcaggtcctgagccccgagagccccttccgcgcacgcggacatgggcggcagctccagggcgcgctgggtggccttggggttgggcgccctggggctgctgtttgctgcgctcggcgttgtcatgatcctcatggtgccctccctcatcaagcagcaggtgctcaagaatgtccgcatagacccgagcagcctgtccttcgggatgtggaaggagatccccgtccctttctacttgtctgtctacttcttcgaagtggtcaacccaaacgaggtcctcaacggccagaagccagtagtccgggagcgtggaccctatgtctacagggagttcagacaaaaggtcaacatcaccttcaatgacaacgacaccgtgtccttcgtggagaaccgcagcctccatttccagcctgacaagtcgcatggctcagagagtgactacattgtactgcctaacatcttggtcctggggggctcgatattgatggagagcaagcctgtgagcctgaagctgatgatgaccttggcgctggtcaccatgggccagcgtgcttttatgaaccgcacagttggtgagatcctgtggggctatgacgatcccttcgtgcattttctcaacacgtacctcccagacatgcttcccataaagggcaaatttggcctgtttgttgggatgaacaactcgaattctggggtcttcactgtcttcacgggcgtccagaatttcagcaggatccatctggtggacaaatggaacggactcagcaagatcgattattggcattcagagcagtgtaacatgatcaatgggacttccgggcagatgtgggcacccttcatgacacccgaatcctcgctggaattcttcagcccggaggcatgcaggtccatgaagctgacctacaacgaatcaagggtgtttgaaggcattcccacgtatcgcttcacggcccccgatactctgtttgccaacgggtccgtctacccacccaacgaaggcttctgcccatgccgagagtctggcattcagaatgtcagcacctgcaggtttggtgcgcctctgtttctctcccacccccacttttacaacgccgaccctgtgttgtcagaagctgttcttggtctgaaccctaacccaaaggagcattccttgttcctagacatccatccggtcactgggatccccatgaactgttctgtgaagatgcagctgagcctctacatcaaatctgtcaagggcatcgggcaaacagggaagatcgagccagtagttctgccgttgctgtggttcgaacagagcggagcaatgggtggcaagcccctgagcacgttctacacgcagctggtgctgatgccccaggttcttcactacgcgcagtatgtgctgctggggcttggaggcctcctgttgctggtgcccatcatctgccaactgcgcagccaggagaaatgctttttgttttggagtggtagtaaaaagggctcccaggataaggaggccattcaggcctactctgagtccctgatgtcaccagctgccaagggcacggtgctgcaagaagccaagctatagggtcctgaagacactataagccccccaaacctgatagcttggtcagaccagccacccagtccctacaccccgcttcttgaggactctctcagcggacagcccaccagtgccatggcctgagcccccagatgtcacacctgtccgcacgcacggcacatggatgcccacgcatgtgcaaaaacaactcagggaccagggacagacctgctgccaagtgagcctgatgggccacaggtgtgctcttctaaatggcctgtgagccaggctgtgggaactctagctgctgtcagcccctcctgtaggagctggccctgcccaggctcctgacttccctcaggaagtctttctgtctttctccatcagtctgaaagccttagttcccacagaggacggatctgtcactcctaggggctgggcatatgtcggcctcttgtgccaaggccaggcaagcagctccaggtcctgaccagtttgcacacacactctggagctgtatctggcgctttttctatcgtctctgctatgtcactgaattaaccactgtacgtggcagaggtggcaggcccctcagggtccttatttttcaggcatggggtcaaagctagaggtatgggccgtctacacccccccgccccccggcatctagtgtacctcaccagagggtattcggaggcccagcatcctgcaaccgaccccttttttctactggaagagaaattttatcatcttttgaaaggaagtcatgactgaagcaataaaccttttcactgattcaacaaaaaaaaaaaaaaa

SEQ ID NO: 6 - DNA, 2759 bp, Homo sapiens
  SR-B1 mRNA
gctcaggccccgcccctgccgccggaatcctgaagcccaaggctgcccgggggcggtccggcggcgccggcgatggggcataaaaccactggccacctgccgggctgctcctgcgtgcgctgccgtcccggatccaccgtgcctctgcggcctgcgtgcccggagtccccgcctgtgtcgtctctgtcgccgtccccgtctcctgccaggcgcggagccctgcgagccgcgggtgggccccaggcgcgcagacatgggctgctccgccaaagcgcgctgggctgccggggcgctgggcgtcgcggggctactgtgcgctgtgctgggcgctgtcatgatcgtgatggtgccgtcgctcatcaagcagcaggtccttaagaacgtgcgcatcgaccccagtagcctgtccttcaacatgtggaaggagatccctatccccttctatctctccgtctacttctttgacgtcatgaaccccagcgagatcctgaagggcgagaagccgcaggtgcgggagcgcgggccctacgtgtacagggagttcaggcacaaaagcaacatcaccttcaacaacaacgacaccgtgtccttcctcgagtaccgcaccttccagttccagccctccaagtcccacggctcggagagcgactacatcgtcatgcccaacatcctggtcttgggtgcggcggtgatgatggagaataagcccatgaccctgaagctcatcatgaccttggcattcaccaccctcggcgaacgtgccttcatgaaccgcactgtgggtgagatcatgtggggctacaaggacccccttgtgaatctcatcaacaagtactttccaggcatgttccccttcaaggacaagttcggattatttgctgagctcaacaactccgactctgggctcttcacggtgttcacgggggtccagaacatcagcaggatccacctcgtggacaagtggaacgggctgagcaaggttgacttctggcattccgatcagtgcaacatgatcaatggaacttctgggcaaatgtggccgcccttcatgactcctgagtcctcgctggagttctacagcccggaggcctgccgatccatgaagctaatgtacaaggagtcaggggtgtttgaaggcatccccacctatcgcttcgtggctcccaaaaccctgtttgccaacgggtccatctacccacccaacgaaggcttctgcccgtgcctggagtctggaattcagaacgtcagcacctgcaggttcagtgcccccttgtttctctcccatcctcacttcctcaacgctgacccggttctggcagaagcggtgactggcctgcaccctaaccaggaggcacactccttgttcctggacatccacccggtcacgggaatccccatgaactgctctgtgaaactgcagctgagcctctacatgaaatctgtcgcaggcattggacaaactgggaagattgagcctgtggtcctgccgctgctctggtttgcagagagcggggccatggagggggagactcttcacacattctacactcagctggtgttgatgcccaaggtgatgcactatgcccagtacgtcctcctggcgctgggctgcgtcctgctgctggtccctgtcatctgccaaatccggagccaagagaaatgctatttattttggagtagtagtaaaaagggctcaaaggataaggaggccattcaggcctattctgaatccctgatgacatcagctcccaagggctctgtgctgcaggaagcaaaactgtagggtcctgaggacaccgtgagccagccaggcctggccgctgggcctgaccggccccccagcccctacaccccgcttctcccggactctcccagcggacagccccccagccccacagcctgagcctcccagctgccatgtgcctgttgcacacctgcacacacgccctggcacacatacacacatgcgtgcaggcttgtgcagacactcagggatggagctgctgctgaagggacttgtagggagaggctcgtcaacaagcactgttctggaaccttctctccacgtggcccacaggcctgaccacaggggctgtgggtcctgcgtccccttcctcgggtgagcctggcctgtcccgttcagccgttgggcccaggcttcctcccctccaaggtgaaacactgcagtcccggtgtggtggctccccatgcaggacgggccaggctgggagtgccgccttcctgtgccaaattcagtggggactcagtgcccaggccctggccacgagctttggccttggtctacctgccaggccaggcaaagcgcctttacacaggcctcggaaaacaatggagtgagcacaagatgccctgtgcagctgcccgagggtctccgcccaccccggccggactttgatccccccgaagtcttcacaggcactgcatcgggttgtctggcgcccttttcctccagcctaaactgacatcatcctatggactgagccggccactctctggccgaagtggccgcaggctgtgcccccgagctgcccccaccccctcacagggtccctcagattataggtgcccaggctgaggtgaagaggcctgggggccctgccttccgggcgctcctggaccctggggcaaacctgtgacccttttctactggaatagaaatgagttttatcatctttgaaaaataattcactcttgaagtaataaacgtttaaaaaaatgggaaaaaaaaaaaaaaaaaa

SEQ ID NO: 7 - DNA, 6982 bp, Mus musculus
  Malat1 mRNA
aggcattcaggcagcgagagcagagcagcgtagagcagcacagctgagctcgtgaggcaggagactcagcccgaggaaatcgcagataagtttttaattaaaaagattgagcagtaaaaagaattagaactctaaacttaagctaatagagtagcttatcgaaatattacttagtcttaataatctaagaagatcttaagagataacatgaaggcttatttaaacagtttgaaaaaggaaatgaggagaaaagtatttgtactgtataatggaggctgaccagagcagtttaggagattgtaaagggaggttttgtgaagttctaaaaggttctagtttgaaggtcggccttgtagattaaaacgaaggttacctaaatagaatctaagtggcatttaaaacagtaaagttgtagagaatagtttgaaaatgaggtgtagttttaaaagattgagaaaagtaggttaagttgacggccgttataaaaatccttcgactggcgcatgtacgtttgaaggcatgagttggaaacagggaagatggaagtgttaggctagccgggcgatggtggcgcacgcctttaatcctagcacttgggaggcagaggcaggcggatttctgagttcgaggccagcctggtctacagagtgagttccaggacagccagggctacacagagaaaccctgtcttgaaaaaacaaaaaggttaggctagtatttggagaaagaagattagaaaatggaagtgaaagacgaagaagacatacaggaaggtgaagaaaaagctgttagagaagataggaaaatagaagacaaagcatctttagaagacagaaaaggtacttaaaggcacaggtagtaggaagccgaagaatagaagatagaaagaagcaagatagaaaaacaaaatggaagttaagacaactttggatgccagcattcaagataggcaaagaagataagattgaggccaaaaggttggataagatataaagtcagaaggaaattatctttaaagccataagttcaaatttctgatggagcgagcagtttagaagagtctttagacagccacatacaagattgaagctagcaatcaaagctactaggactgaagtaaaaagttaaggcagaatgcctttgaagagttagaagaatattaaaagccttaacttgtagcttaattttgcttgatgacaaaaggacttttgataacagtttcaagattgtcagcattttgcattggacttgagctgaggtgcttttaaaatcctaacgactagcattggcagctgacccaggtctacacagaagtgcattcagtgaactaggaagacaggagcggcagacaggagtcccgaagccagtttggtgaagctaggaaggactgaggagccagcagcagcagtgcatggtgaagatagcccaggaaagagtgcggttcggtggaggaagctaggaagaaggagccatacggatgtggtggtgaagctgggaaagggttccaggatggtggagcgagagcgagttggtgatgaagctagctggcggcttggcttgtcaactgcgcggaggaggcgagcaggcattgtggagaggatagatagcggctcctagaccagcatgccagtgtgcaagaaaggctgcagggagagcatgcggtgcggtaacattccttgaggtcggcaacatggtggtggttttctgtaacttggatggtaacttgtttactttgtcttaatagttatgggggagttgtaggcttctgtgtaaagagatatatctggggctgtatgtaggcctttgcgggtgttgtaggtttttctttttcagggttatgtcctcttgcatcttgtcagaagcttttgagggctgactgccaaggcccagaaagaagaatggtagatggcaagttgtctttaaccgctcagaggggaatgaatggtagagccagcacaacctcccagttttgtaagacgttgtagtttgaacagatgacctaccacaagcctcactcctgtgtaggggaggtaattgggcaaagtgcttttgggggaatgggggcaaaatatattttgagttcttttccccttaggtctgtctagaatcctaaaggcagatgactcaagggaaccagaaaaaaggaaatccactctcaggataagcagagctcgccaggtttacagtttgtaggaagtagaggatggatgctagctttcacactgagtgtggaggagctggccatggcggaattgctggtagtttactctttccccctcccttaatgagatttgtaaaatcctaaacacttttacttgaaatatttgggagtggtcttaacagggaggagtgggtgggggaaacgttttttttctaagattttccacagatgctatagttgtgttgacacactgggttagagaaggcgtgtactgctatgctgttggcacgacaccttcagggactggagctgccttttgtccttggaagagttttcccagttgccgctgaagtcagcacagtgcggctttggttcacagtcacctcaggagaacctcaggagcttggctaggccagaggttgaagttaagttttacagcaccgtgatttaaaatatttcattaaaggggaggggtaaaacttagttggctgtggccttgtgtttgggtgggtgggggtgttaggtaattgtttagtttatgatttcagataatcataccagagaacttaaatatttggaaaaacaggaaatctcagctttcaagttggcaagtaactcccaatccagtttttgcttcttttttcctttttctttttttgaggcgggcagctaaggaaggttggttcctctgccggtccctcgaaagcgtagggcttgggggttggtctggtccactgggatgatgtgatgctacagtggggactcttctgaagctgttggatgaatatagattgtagtgtgtggttctcttttgaaatttttttcaggtgacttaatgtatcttaataactactataggaacaaaggaagtggctttaatgaccctgaaggaatttcttctggtgatagcttttatattatcaagtaagagatactatctcagttttgtataagcaagtctttttcctagtgtaggagaaatgattttccttgtgactaaacaagatgtaaaggtatgctttttttcttcttgtgcattgtatacttgtgtttatttgtaacttataatttaagaattatgataattcagcctgaatgtcttttagagggtgggcttttgttgatgagggaggggaaacctttttttttctgtagacctttttcagataacaccatctgagtcataaccagcctggcagtgtgatgacgtagatgcagagggagcagctccttggtgaatgagtgataagtaaaggcagaaaaaataatgtcatgtctccatggggaatgagcatgagccagagattgttcctactgatgaaaagctgcatatgcaaaaatttaagcaaatgaaagcaaccagtataaagttatggcaatacctttaaaagttatggcttatctaccaagctttatccacaaaagtaaagaattgatgaaaaacagtgaagatcaaatgttcatctcaaaactgcttttacaaaagcagaatagaaatgaagtgaaaatgctgcattaagcctggagtaaaaagaagctgagcttgttgagatgagtgggatcgagcggctgcgaggcggtgcagtgtgccaatgtttcgtttgcctcagacaggtttctcttcataagcagaagagttgcttcattccatctcggagcaggaaacagcagactgctgttgacagataagtgtaacttggatctgcagtattgcatgttagggatagataagtgccttttttctctttttccaaaaagacctgtagagctgttgaatgtttgcagctggcccctcttaggcagttcagaattttgagtagttttcccatccagcctcttaaaaattcctaagccttgcaccgatgggctttcatgatgggatagctaataggcttttgcatcgtaaacttcaacacaaaagcctacatgattaatgcctactttaattacattgcttacaagattaaggaatctttatcttgaagaccccatgaaagggatcattatgtgctgaaaattagatgttcatattgctaaaatttaaatgtgctccaatgtacttgtgcttaaaatcattaaattatacaaattaataaaatacttcactagagaatgtatgtatttagaaggctgtctccttatttaaataaagtcttgtttgttgtctgtagttagtgtgggcaattttggggggatgttcttctctaatcttttcagaaacttgacttcgaacacttaagtggaccagatcaggatttgagccagaagaccgaaattaactttaaggcaggaaagacaaattttattctccatgcagtgatgagcatttaataattgcaggcctggcatagaggccgtctaactaaggactaagtaccttaggcaggtgggagatgatggtcagagtaaaaggtaactacatattttgtttccagaaagtcaggggtctaatttgaccatggctaaacatctagggtaagacacttttcccccacatttccaaatatgcatgttgagtttaaatgcttacgatcatctcatccactttagccttttgtcacctcacttgagccacgagtggggtcaggcatgtgggtttaaagagttttcctttgcagagcctcatttcatccttcatggagctgctcaggactttgcatataagcgcttgcctctgtcttctgttctgctagtgagtgtgtgatgtgagaccttgcagtgagtttgtttttcctggaatgtggagggagggggggatggggcttacttgttctagctttttttttacagaccacacagaatgcaggtgtcttgacttcaggtcatgtctgttctttggcaagtaatatgtgcagtactgttccaatctgctgctattagaatgcattgtgacgcgactggagtatgattaaagaaagttgtgtttccccaagtgtttggagtagtggttgttggaggaaaagccatgagtaacaggctgagtgttgaggaaatggctctctgcagctttaagtaacccgtgtttgtgattggagccgagtccctttgctgtgctgccttaggtaaatgtttttgttcatttctggtgaggggggttgggagcactgaagcctttagtctcttccagattcaacttaaaatctgacaagaaataaatcagacaagcaacattcttgaagaaattttaactggcaagtggaaatgttttgaacagttccgtggtctttagtgcattatctttgtgtaggtgttctctctcccctcccttggtcttaattcttacatgcaggaacattgacaacagcagacatctatctattcaaggggccagagaatccagacccagtaaggaaaaatagcccatttactttaaatcgataagtgaagcagacatgccattttcagtgtggggattgggaagccctagttctttcagatgtacttcagactgtagaaggagcttccagttgaattgaaattcaccagtggacaaaatgaggacaacaggtgaacgagccttttcttgtttaagattagctactggtaatctagtgttgaatcctctccagcttcatgctggagcagctagcatgtgatgtaatgttggccttggggtggaggggtgaggtgggcgctaagcctttttttaagatttttcaggtacccctcactaaaggcactgaaggcttaatgtaggacagcggagccttcctgtgtggcaagaatcaagcaagcagtattgtatcgagaccaaagtggtatcatggtcggttttgattagcagtggggactaccctaccgtaacaccttgttggaattgaagcatccaaagaaaatacttgagaggccctgggcttgttttaacatctggaaaaaaggctgtttttatagcagcggttaccagcccaaacctcaagttgtgcttgcaggggagggaaaagggggaaagcgggcaaccagtttccccagcttttccagaatcctgttacaaggtctccccacaagtgatttctctgccacatcgccaccatgggcctttggcctaatcacagacccttcacccctcaccttgatgcagccagtagctggatccttgaggtcacgttgcatatcggtttcaaggtaaccatggtgccaaggtcctgtgggttgcaccagaaaaggccatcaattttccccttgcctgtaatttaacattaaaaccatagctaagatgttttatacatagcacctatgcagagtaaacaaaccagtatgggtatagtatgtttgataccagtgctgggtgggaatgtaggaagtcggatgaaaagcaagcctttgtaggaagttgttggggtgggattgcaaaaattctctgctaagactttttcaggtggacataacagacttggccaagctagcatcttagtggaagcagattcgtcagtagggttgtaaaggtttttcttttcctgagaaaacaaccttttgttttctcaggttttgctttttggcctttccctagctttaaaaaaaaaaaagcaaaagacgctggtggctggcactcctggtttccaggacggggttcaagtccctgcggtgtctttgcttgactcttatatcatgaggccattacatttttcttggagggttctaaaggctctgggtatggtagctgatatcactggaacactccccagcctcagtgttgaactcttgataattaactgcattgtctttcaggttatgcccaattcgtcttattacctctgagtcgacacacctcctactatttattgaatactttgattttatgaaataaaaactaaatatctctca

SEQ ID NO: 8 - DNA, 8758 bp, Homo sapiens
  Malat1 mRNA
gtaaaggactggggccccgcaactggcctctcctgccctcttaagcgcagcgccattttagcaacgcagaagcccggcgccgggaagcctcagctcgcctgaaggcaggtcccctctgacgcctccgggagcccaggtttcccagagtccttgggacgcagcgacgagttgtgctgctatcttagctgtccttataggctggccattccaggtggtggtatttagataaaaccactcaaactctgcagtttggtcttggggtttggaggaaagcttttatttttcttcctgctccggttcagaaggtctgaagctcatacctaaccaggcataacacagaatctgcaaaacaaaaacccctaaaaaagcagacccagagcagtgtaaacacttctgggtgtgtccctgactggctgcccaaggtctctgtgtcttcggagacaaagccattcgcttagttggtctactttaaaaggccacttgaactcgctttccatggcgatttgccttgtgagcactttcaggagagcctggaagctgaaaaacggtagaaaaatttccgtgcgggccgtggggggctggcggcaactggggggccgcagatcagagtgggccactggcagccaacggcccccggggctcaggcggggagcagctctgtggtgtgggattgaggcgttttccaagagtgggttttcacgtttctaagatttcccaagcagacagcccgtgctgctccgatttctcgaacaaaaaagcaaaacgtgtggctgtcttgggagcaagtcgcaggactgcaagcagttgggggagaaagtccgccattttgccacttctcaaccgtccctgcaaggctggggctcagttgcgtaatggaaagtaaagccctgaactatcacactttaatcttccttcaaaaggtggtaaactatacctactgtccctcaagagaacacaagaagtgctttaagaggtattttaaaagttccgggggttttgtgaggtgtttgatgacccgtttaaaatatgatttccatgtttcttttgtctaaagtttgcagctcaaatctttccacacgctagtaatttaagtatttctgcatgtgtagtttgcattcaagttccataagctgttaagaaaaatctagaaaagtaaaactagaacctatttttaaccgaagaactactttttgcctccctcacaaaggcggcggaaggtgatcgaattccggtgatgcgagttgttctccgtctataaatacgcctcgcccgagctgtgcggtaggcattgaggcagccagcgcaggggcttctgctgagggggcaggcggagcttgaggaaaccgcagataagtttttttctctttgaaagatagagattaatacaactacttaaaaaatatagtcaataggttactaagatattgcttagcgttaagtttttaacgtaattttaatagcttaagattttaagagaaaatatgaagacttagaagagtagcatgaggaaggaaaagataaaaggtttctaaaacatgacggaggttgagatgaagcttcttcatggagtaaaaaatgtatttaaaagaaaattgagagaaaggactacagagccccgaattaataccaatagaagggcaatgcttttagattaaaatgaaggtgacttaaacagcttaaagtttagtttaaaagttgtaggtgattaaaataatttgaaggcgatcttttaaaaagagattaaaccgaaggtgattaaaagaccttgaaatccatgacgcagggagaattgcgtcatttaaagcctagttaacgcatttactaaacgcagacgaaaatggaaagattaattgggagtggtaggatgaaacaatttggagaagatagaagtttgaagtggaaaactggaagacagaagtacgggaaggcgaagaaaagaatagagaagatagggaaattagaagataaaaacatacttttagaagaaaaaagataaatttaaacctgaaaagtaggaagcagaagaaaaaagacaagctaggaaacaaaaagctaagggcaaaatgtacaaacttagaagaaaattggaagatagaaacaagatagaaaatgaaaatattgtcaagagtttcagatagaaaatgaaaaacaagctaagacaagtattggagaagtatagaagatagaaaaatataaagccaaaaattggataaaatagcactgaaaaaatgaggaaattattggtaaccaatttattttaaaagcccatcaatttaatttctggtggtgcagaagttagaaggtaaagcttgagaagatgagggtgtttacgtagaccagaaccaatttagaagaatacttgaagctagaaggggaagttggttaaaaatcacatcaaaaagctactaaaaggactggtgtaatttaaaaaaaactaaggcagaaggcttttggaagagttagaagaatttggaaggccttaaatatagtagcttagtttgaaaaatgtgaaggactttcgtaacggaagtaattcaagatcaagagtaattaccaacttaatgtttttgcattggactttgagttaagattattttttaaatcctgaggactagcattaattgacagctgacccaggtgctacacagaagtggattcagtgaatctaggaagacagcagcagacaggattccaggaaccagtgtttgatgaagctaggactgaggagcaagcgagcaagcagcagttcgtggtgaagataggaaaagagtccaggagccagtgcgatttggtgaaggaagctaggaagaaggaaggagcgctaacgatttggtggtgaagctaggaaaaaggattccaggaaggagcgagtgcaatttggtgatgaaggtagcaggcggcttggcttggcaaccacacggaggaggcgagcaggcgttgtgcgtagaggatcctagaccagcatgccagtgtgccaaggccacagggaaagcgagtggttggtaaaaatccgtgaggtcggcaatatgttgtttttctggaacttacttatggtaaccttttatttattttctaatataatgggggagtttcgtactgaggtgtaaagggatttatatggggacgtaggccgatttccgggtgttgtaggtttctctttttcaggcttatactcatgaatcttgtctgaagcttttgagggcagactgccaagtcctggagaaatagtagatggcaagtttgtgggttttttttttttacacgaatttgaggaaaaccaaatgaatttgatagccaaattgagacaatttcagcaaatctgtaagcagtttgtatgtttagttggggtaatgaagtatttcagttttgtgaatagatgacctgtttttacttcctcaccctgaattcgttttgtaaatgtagagtttggatgtgtaactgaggcgggggggagttttcagtatttttttttgtgggggtgggggcaaaatatgttttcagttctttttcccttaggtctgtctagaatcctaaaggcaaatgactcaaggtgtaacagaaaacaagaaaatccaatatcaggataatcagaccaccacaggtttacagtttatagaaactagagcagttctcacgttgaggtctgtggaagagatgtccattggagaaatggctggtagttactcttttttccccccacccccttaatcagactttaaaagtgcttaaccccttaaacttgttattttttacttgaagcattttgggatggtcttaacagggaagagagagggtgggggagaaaatgtttttttctaagattttccacagatgctatagtactattgacaaactgggttagagaaggagtgtaccgctgtgctgttggcacgaacaccttcagggactggagctgcttttatccttggaagagtattcccagttgaagctgaaaagtacagcacagtgcagctttggttcatattcagtcatctcaggagaacttcagaagagcttgagtaggccaaatgttgaagttaagttttccaataatgtgacttcttaaaagttttattaaaggggaggggcaaatattggcaattagttggcagtggcctgttacggttgggattggtggggtgggtttaggtaattgtttagtttatgattgcagataaactcatgccagagaacttaaagtcttagaatggaaaaagtaaagaaatatcaacttccaagttggcaagtaactcccaatgatttagtttttttccccccagtttgaattgggaagctgggggaagttaaatatgagccactgggtgtaccagtgcattaatttgggcaaggaaagtgtcataatttgatactgtatctgttttccttcaaagtatagagcttttggggaaggaaagtattgaactgggggttggtctggcctactgggctgacattaactacaattatgggaaatgcaaaagttgtttggatatggtagtgtgtggttctcttttggaatttttttcaggtgatttaataataatttaaaactactatagaaactgcagagcaaaggaagtggcttaatgatcctgaagggatttcttctgatggtagcttttgtattatcaagtaagattctattttcagttgtgtgtaagcaagtttttttttagtgtaggagaaatacttttccattgtttaactgcaaaacaagatgttaaggtatgcttcaaaaattttgtaaattgtttattttaaacttatctgtttgtaaattgtaactgattaagaattgtgatagttcagcttgaatgtctcttagagggtgggcttttgttgatgagggaggggaaactttttttttttctatagacttttttcagataacatcttctgagtcataaccagcctggcagtatgatggcctagatgcagagaaaacagctccttggtgaattgataagtaaaggcagaaaagattatatgtcatacctccattggggaataagcataaccctgagattcttactactgatgagaacattatctgcatatgccaaaaaattttaagcaaatgaaagctaccaatttaaagttacggaatctaccattttaaagttaattgcttgtcaagctataaccacaaaaataatgaattgatgagaaatacaatgaagaggcaatgtccatctcaaaatactgcttttacaaaagcagaataaaagcgaaaagaaatgaaaatgttacactacattaatcctggaataaaagaagccgaaataaatgagagatgagttgggatcaagtggattgaggaggctgtgctgtgtgccaatgtttcgtttgcctcagacaggtatctcttcgttatcagaagagttgcttcatttcatctgggagcagaaaacagcaggcagctgttaacagataagtttaacttgcatctgcagtattgcatgttagggataagtgcttatttttaagagctgtggagttcttaaatatcaaccatggcactttctcctgaccccttccctaggggatttcaggattgagaaatttttccatcgagcctttttaaaattgtaggacttgttcctgtgggcttcagtgatgggatagtacacttcactcagaggcatttgcatctttaaataatttcttaaaagcctctaaagtgatcagtgccttgatgccaactaaggaaatttgtttagcattgaatctctgaaggctctatgaaaggaatagcatgatgtgctgttagaatcagatgttactgctaaaatttacatgttgtgatgtaaattgtgtagaaaaccattaaatcattcaaaataataaactatttttattagagaatgtatacttttagaaagctgtctccttatttaaataaaatagtgtttgtctgtagttcagtgttggggcaatcttgggggggattcttctctaatctttcagaaactttgtctgcgaacactctttaatggaccagatcaggatttgagcggaagaacgaatgtaactttaaggcaggaaagacaaattttattcttcataaagtgatgagcatataataattccaggcacatggcaatagaggccctctaaataaggaataaataacctcttagacaggtgggagattatgatcagagtaaaaggtaattacacattttatttccagaaagtcaggggtctataaattgacagtgattagagtaatactttttcacatttccaaagtttgcatgttaactttaaatgcttacaatcttagagtggtaggcaatgttttacactattgaccttatatagggaagggagggggtgcctgtggggttttaaagaattttcctttgcagaggcatttcatccttcatgaagccattcaggattttgaattgcatatgagtgcttggctcttccttctgttctagtgagtgtatgagaccttgcagtgagtttatcagcatactcaaaatttttttcctggaatttggagggatgggaggagggggtggggcttacttgttgtagctttttttttttttacagacttcacagagaatgcagttgtcttgacttcaggtctgtctgttctgttggcaagtaaatgcagtactgttctgatcccgctgctattagaatgcattgtgaaacgactggagtatgattaaaagttgtgttccccaatgcttggagtagtgattgttgaaggaaaaaatccagctgagtgataaaggctgagtgttgaggaaatttctgcagttttaagcagtcgtatttgtgattgaagctgagtacattttgctggtgtatttttaggtaaaatgctttttgttcatttctggtggtgggaggggactgaagcctttagtcttttccagatgcaaccttaaaatcagtgacaagaaacattccaaacaagcaacagtcttcaagaaattaaactggcaagtggaaatgtttaaacagttcagtgatctttagtgcattgtttatgtgtgggtttctctctcccctcccttggtcttaattcttacatgcaggaacactcagcagacacacgtatgcgaagggccagagaagccagacccagtaagaaaaaatagcctatttactttaaataaaccaaacattccattttaaatgtggggattgggaaccactagttctttcagatggtattcttcagactatagaaggagcttccagttgaattcaccagtggacaaaatgaggaaaacaggtgaacaagctttttctgtatttacatacaaagtcagatcagttatgggacaatagtattgaatagatttcagctttatgctggagtaactggcatgtgagcaaactgtgttggcgtgggggtggaggggtgaggtgggcgctaagcctttttttaagatttttcaggtacccctcactaaaggcaccgaaggcttaaagtaggacaaccatggagccttcctgtggcaggagagacaacaaagcgctattatcctaaggtcaagagaagtgtcagcctcacctgatttttattagtaatgaggacttgcctcaactccctctttctggagtgaagcatccgaaggaatgcttgaagtacccctgggcttctcttaacatttaagcaagctgtttttatagcagctcttaataataaagcccaaatctcaagcggtgcttgaaggggagggaaagggggaaagcgggcaaccacttttccctagcttttccagaagcctgttaaaagcaaggtctccccacaagcaacttctctgccacatcgccaccccgtgccttttgatctagcacagacccttcacccctcacctcgatgcagccagtagcttggatccttgtgggcatgatccataatcggtttcaaggtaacgatggtgtcgaggtctttggtgggttgaactatgttagaaaaggccattaatttgcctgcaaattgttaacagaagggtattaaaaccacagctaagtagctctattataatacttatccagtgactaaaaccaacttaaaccagtaagtggagaaataacatgttcaagaactgtaatgctgggtgggaacatgtaacttgtagactggagaagataggcatttgagtggctgagagggcttttgggtgggaatgcaaaaattctctgctaagactttttcaggtgaacataacagacttggccaagctagcatcttagcggaagctgatctccaatgctcttcagtagggtcatgaaggtttttcttttcctgagaaaacaacacgtattgttttctcaggttttgctttttggcctttttctagcttaaaaaaaaaaaaagcaaaagatgctggtggttggcactcctggtttccaggacggggttcaaatccctgcggcgtctttgctttgactactaatctgtcttcaggactctttctgtatttctccttttctctgcaggtgctagttcttggagttttggggaggtgggaggtaacagcacaatatctttgaactatatacatccttgatgtataatttgtcaggagcttgacttgattgtatattcatatttacacgagaacctaatataactgccttgtctttttcaggtaatagcctgcagctggtgttttgagaagccctactgctgaaaacttaacaattttgtgtaataaaaatggagaagctctaaattgttgtggttcttttgtgaataaaaaaatcttgattggggaaaaaaaaa

SEQ ID NO: 9 - DNA, 2761 bp, Mus musculus
  DMPK mRNA
gaactggccagagagacccaagggatagtcagggacgggcagacatgcagctagggttctggggcctggacaggggcagccaggccctgtgacgggaagaccccgagctccggcccggggaggggccatggtgttgcctgcccaacatgtcagccgaagtgcggctgaggcagctccagcagctggtgctggacccaggcttcctgggactggagcccctgctcgaccttctcctgggcgtccaccaggagctgggtgcctctcacctagcccaggacaagtatgtggccgacttcttgcagtgggtggagcccattgcagcaaggcttaaggaggtccgactgcagagggatgattttgagattttgaaggtgatcgggcgtggggcgttcagcgaggtagcggtggtgaagatgaaacagacgggccaagtgtatgccatgaagattatgaataagtgggacatgctgaagagaggcgaggtgtcgtgcttccgggaagaaagggatgtattagtgaaaggggaccggcgctggatcacacagctgcactttgccttccaggatgagaactacctgtacctggtcatggaatactacgtgggcggggacctgctaacgctgctgagcaagtttggggagcggatccccgccgagatggctcgcttctacctggccgagattgtcatggccatagactccgtgcaccggctgggctacgtgcacagggacatcaaaccagataacattctgctggaccgatgtgggcacattcgcctggcagacttcggctcctgcctcaaactgcagcctgatggaatggtgaggtcgctggtggctgtgggcaccccggactacctgtctcctgagattctgcaggccgttggtggagggcctggggcaggcagctacgggccagagtgtgactggtgggcactgggcgtgttcgcctatgagatgttctatgggcagacccccttctacgcggactccacagccgagacatatgccaagattgtgcactacagggaacacttgtcgctgccgctggcagacacagttgtccccgaggaagctcaggacctcattcgtgggctgctgtgtcctgctgagataaggctaggtcgaggtggggcaggtgatttccagaaacatcctttcttctttggccttgattgggagggtctccgagacagtgtacccccctttacaccagacttcgagggtgccacggacacatgcaatttcgatgtggtggaggaccggctcactgccatggtgagcgggggcggggagacgctgtcagacatgcaggaagacatgccccttggggtgcgcctgcccttcgtgggctactcctactgctgcatggccttcagagacaatcaggtcccggaccccacccctatggaactagaggccctgcagttgcctgtgtcagacttgcaagggcttgacttgcagcccccagtgtccccaccggatcaagtggctgaagaggctgacctagtggctgtccctgcccctgtggctgaggcagagaccacggtaacgctgcagcagctccaggaagccctggaagaagaggttctcacccggcagagcctgagccgcgagctggaggccatccggaccgccaaccagaacttctccagccaactacaggaggccgaggtccgaaaccgagacctggaggcgcatgttcggcagctacaggaacggatggagatgctgcaggccccaggagccgcagccatcacgggggtccccagtccccgggccacggatccaccttcccatctagatggccccccggccgtggctgtgggccagtgcccgctggtggggccaggccccatgcaccgccgtcacctgctgctccctgccaggatccctaggcctggcctatccgaggcgcgttgcctgctcctgttcgccgctgctctggctgctgccgccacactgggctgcactgggttggtggcctataccggcggtctcaccccagtctggtgtttcccgggagccaccttcgccccctgaaccctaagactccaagccatctttcatttaggcctcctaggaaggtcgagcgaccagggagcgacccaaagcgtctctgtgcccatcgcgccccccccccccccccaccgctccgctccacacttctgtgagcctgggtccccacccagctccgctcctgtgatccaggcctgccacctggcggccggggagggaggaacagggctcgtgcccagcacccctggttcctgcagagctggtagccaccgctgctgcagcagctgggcattcgccgaccttgctttactcagccccgacgtggatgggcaaactgctcagctcatccgatttcactttttcactctcccagccatcagttacaagccataagcatgagccccctatttccagggacatcccattcccatagtgatggatcagcaagacctctgccagcacacacggagtctttggcttcggacagcctcactcctgggggttgctgcaactccttccccgtgtacacgtctgcactctaacaacggagccacagctgcactcccccctcccccaaagcagtgtgggtatttattgatcttgttatctgactcactgacagactccgggacccacgttttagatgcattgagactcgacattcctcggtatttattgtctgtccccacctacgacctccactcccgacccttgcgaataaaatacttctggtctgccctaaa

SEQ ID NO: 10 - DNA, 3243 bp, Homo sapiens
  DMPK mRNA
gccacaagcctccaccccagctggtcccccacccaggctgcccagtttaacattcctagtcataggaccttgacttctgagaggcctgattgtcatctgtaaataaggggtaggactaaagcactcctcctggaggactgagagatgggctggaccggagcacttgagtctgggatatgtgaccatgctacctttgtctccctgtcctgttccttcccccagccccaaatccagggttttccaaagtgtggttcaagaaccacctgcatctgaatctagaggtactggatacaaccccacgtctgggccgttacccaggacattctacatgagaacgtgggggtggggccctggctgcacctgaactgtcacctggagtcagggtggaaggtggaagaactgggtcttatttccttctccccttgttctttagggtctgtccttctgcagactccgttaccccaccctaaccatcctgcacacccttggagccctctgggccaatgccctgtcccgcaaagggcttctcaggcatctcacctctatgggagggcatttttggcccccagaaccttacacggtgtttatgtggggaagcccctgggaagcagacagtcctagggtgaagctgagaggcagagagaaggggagacagacagagggtggggctttcccccttgtctccagtgccctttctggtgaccctcggttcttttcccccaccacccccccagcggagcccatcgtggtgaggcttaaggaggtccgactgcagagggacgacttcgagattctgaaggtgatcggacgcggggcgttcagcgaggtagcggtagtgaagatgaagcagacgggccaggtgtatgccatgaagatcatgaacaagtgggacatgctgaagaggggcgaggtgtcgtgcttccgtgaggagagggacgtgttggtgaatggggaccggcggtggatcacgcagctgcacttcgccttccaggatgagaactacctgtacctggtcatggagtattacgtgggcggggacctgctgacactgctgagcaagtttggggagcggattccggccgagatggcgcgcttctacctggcggagattgtcatggccatagactcggtgcaccggcttggctacgtgcacagggacatcaaacccgacaacatcctgctggaccgctgtggccacatccgcctggccgacttcggctcttgcctcaagctgcgggcagatggaacggtgcggtcgctggtggctgtgggcaccccagactacctgtcccccgagatcctgcaggctgtgggcggtgggcctgggacaggcagctacgggcccgagtgtgactggtgggcgctgggtgtattcgcctatgaaatgttctatgggcagacgcccttctacgcggattccacggcggagacctatggcaagatcgtccactacaaggagcacctctctctgccgctggtggacgaaggggtccctgaggaggctcgagacttcattcagcggttgctgtgtcccccggagacacggctgggccggggtggagcaggcgacttccggacacatcccttcttctttggcctcgactgggatggtctccgggacagcgtgcccccctttacaccggatttcgaaggtgccaccgacacatgcaacttcgacttggtggaggacgggctcactgccatggtgagcgggggcggggagacactgtcggacattcgggaaggtgcgccgctaggggtccacctgccttttgtgggctactcctactcctgcatggccctcagggacagtgaggtcccaggccccacacccatggaactggaggccgagcagctgcttgagccacacgtgcaagcgcccagcctggagccctcggtgtccccacaggatgaaacagctgaagtggcagttccagcggctgtccctgcggcagaggctgaggccgaggtgacgctgcgggagctccaggaagccctggaggaggaggtgctcacccggcagagcctgagccgggagatggaggccatccgcacggacaaccagaacttcgccagtcaactacgcgaggcagaggctcggaaccgggacctagaggcacacgtccggcagttgcaggagcggatggagttgctgcaggcagagggagccacagctgtcacgggggtccccagtccccgggccacggatccaccttcccatctagatggccccccggccgtggctgtgggccagtgcccgctggtggggccaggccccatgcaccgccgccacctgctgctccctgccagggtccctaggcctggcctatcggaggcgctttccctgctcctgttcgccgttgttctgtctcgtgccgccgccctgggctgcattgggttggtggcccacgccggccaactcaccgcagtctggcgccgcccaggagccgcccgcgctccctgaaccctagaactgtcttcgactccggggccccgttggaagactgagtgcccggggcacggcacagaagccgcgcccaccgcctgccagttcacaaccgctccgagcgtgggtctccgcccagctccagtcctgtgatccgggcccgccccctagcggccggggagggaggggccgggtccgcggccggcgaacggggctcgaagggtccttgtagccgggaatgctgctgctgctgctgctgctgctgctgctgctgctgctgctgctgctgctgctgctgctggggggatcacagaccatttctttctttcggccaggctgaggccctgacgtggatgggcaaactgcaggcctgggaaggcagcaagccgggccgtccgtgttccatcctccacgcacccccacctatcgttggttcgcaaagtgcaaagctttcttgtgcatgacgccctgctctggggagcgtctggcgcgatctctgcctgcttactcgggaaatttgcttttgccaaacccgctttttcggggatcccgcgcccccctcctcacttgcgctgctctcggagccccagccggctccgcccgcttcggcggtttggatatttattgacctcgtcctccgactcgctgacaggctacaggacccccaacaaccccaatccacgttttggatgcactgagaccccgacattcctcggtatttattgtctgtccccacctaggacccccacccccgaccctcgcgaataaaaggccctccatctgcccaaagctctgga

SEQ ID NO: 11 - DNA, 41 bp, Artificial
  synthetic
  DNA/RNA molecule
gcauucagugaacuaguucaagagactagttcactgaatgc

SEQ ID NO: 12 - DNA, 30 bp, Artificial
  synthetic
ctccaacatcaaggaagatggcatttctag

SEQ ID NO: 13 - DNA, 25 bp, Artificial
  synthetic
gttgcctccggttctgaaggtgttc

SEQ ID NO: 14 - DNA, 21 bp, Artificial
  synthetic
cctccggttctgaaggtgttc

SEQ ID NO: 15 - DNA, 22 bp, Artificial
  synthetic
caatgccatcctggagttcctg

SEQ ID NO: 16 - DNA, 16 bp, Artificial
  synthetic
  misc_feature (1)..(3): LNA
  misc_feature (14)..(16): LNA
ctagttcactgaatgc

SEQ ID NO: 17 - RNA, 16 nt, Artificial
  synthetic
  misc_feature (1)..(3): 2'-O-Me RNA
  misc_feature (14)..(16): 2'-O-Me RNA
gcauucagugaacuag

SEQ ID NO: 18 - RNA, 25 nt, Artificial
  synthetic
  misc_feature (1)..(3), (23)..(25): 2'-O-Me RNA
  misc_feature (4)..(22): DNA
auuucagguaagccgagguuuggcc

SEQ ID NO: 19 - RNA, 25 nt, Artificial
  synthetic
  misc_feature (1)..(25): 2'-O-Me RNA
auuucagguaagccgagguuuggcc